European Patent Specification EP 3 839 055 B1, published August 23, 2023. Title: YEAST PROMOTERS FOR PROTEIN EXPRESSION. Applicant: BIOGRAMMATICS, INC. Application not yet assigned. The sequence listing filed with the application follows.

SEQUENCE LISTING (37 sequences)

SEQ ID NO: 1 - DNA, 1000 bp, Pichia pastoris
attgttgtgaatactctccttcatttggatttcttggacttcggactctcttgatctctcttcgaaagttttaactctgttcatgtataattttacccgctgtaggtcgctcataataccatgagtatgcacatcttttactccattaactttcaggtatgcaaaatacaatgaagatagtatatagctcaaagaatttagcattttgcattgatctaattgtgacattttctctatgatatcatctagcttcttaaactcgagaatctcgtccaacgaggcagaaacattgtccagtcttacgtcaagattattcacgagtttctggaccgtatcaacgttttccatcttaagattacagtaagtatcgtccttttgaactgcaaaggtagaaaagttaatttttgatttggtagtacactatgaaacttgctcaccccaatctttcctcctgacaggttgatctttatccctctactaaattgccccaagtgtatcaagtagactagatctcgcgaaagaacagcctaataaactccgaagcatgatggcctctatccggaaaacgttaagagatgtggcaacaggagggcacatagaatttttaaagacgctgaagaatgctatcatagtccgtaaaaatgtgatagtactttgtttagtgcgtacgccacttattcggggccaatagctaaacccaggtttgctggcagcaaattcaactgtagattgaatctctctaacaataatggtgttcaatcccctggctggtcacggggaggactatcttgcgtgatccgcttggaaaatgttgtgtatccctttctcaattgcggaaagcatctgctacttcccataggcaccagttacccaattgatatttccaaaaaagattaccatatgttcatctagaagtataaatacaagtggacattcaatgaatatttcattcaattagtcattgacactttcatcaacttactacgtcttattcaacaat

SEQ ID NO: 2 - DNA, 1000 bp, Pichia pastoris
gtcaactgcgtactcttttgtcgaatggactactgaatctgcctcgatagccactataggaaggtccatagaggccagtttttcaactagtcttggtggaaagaaaccgacaaagcctttcatggagtcaccgatactgaaaggttcaaacaaagaatgcttgggtagtctcttaatacccatggcaacgaaaaaggggtcttcattgttcaacatgaattcgtatccacctttaatgtagtcataaagctgctgaagttccgaatcagtgatggaactgtctacagtgacaatataggagttctcaatcaccttatatccagtcgaatatatctggatagggtcgggtctcactgtggaagattcaaatgggttagatccctgtaatttcagcgatggagactcagtatgatggggcaaggaaaacggcaattggatattcaattggtcaagagatggtatcaaaagcgagtgtgccagggtagccacggtagccactgatgctaatctgataattttcatttctggagtgtcaaaacagtagtgataaaaggctatgaaggaggttgtctaggggctcgcggaggaaagtgattcaaacagacctgccaaaaagagaaaaaagagggaatccctgttctttccaatggaaatgacgtaactttaacttgaaaaataccccaaccagaagggttcaaactcaacaaggattgcgtaattcctacaagtagcttagagctgggggagagacaactgaaggcagcttaacgataacgcggggggattggtgcacgactcgaaaggaggtatcttagtcttgtaacctcttttttccagaggctattcaagattcataggcgatatcgatgtggagaagggtgaacaatataaaaggctggagagatgtcaatgaagcagctggatagatttcaaattttctagatttcagagtaatcgcacaaaacgaaggaatcccaccaagcaaaaaaaaaaaatctaa

SEQ ID NO: 3 - DNA, 1000 bp, Pichia pastoris
tgctgttttgggctcgtacggatgtttcttaggtccgatgattggtgttatgacttgtgactactacttcgtacgtcatcagaaactcaagctgacagacctctacaaagccgacaagagttctatttactggttctacaaaggattcaactggagaggtttcgttgcctggatttgcggttttactccaggtattacagggtttcctagcgtcaaccccaacttgactggggttcctacagcctgtatcaagatgttctacatttcgtttatcattggttacccgatcggattcttagttcatctggcactcaataagctattccctccaccaggtcttggtgaagtcgatgagtatgactactaccactctttcaccgaaaaggaagcactgaaattaggaatggcccctagttccgagttggacagagtcagcaccgatgacccgatcaatattccttacgacgagaagtctttaggctaatgtagttaaatagttaatcgaaacaatcgtgtatcctctttatcgtaccagcgggattcgctgcttggatgggtgactcctgtccagttgactcaaagtagtcaaaataggcctggagacccttaacaggtcgatgagtagcctactatgagaaaacccctcaccacaactggactataaaagggcacgtcaatccccaaagcaactcttttctttcatccctactttattactttatcctttgatcttcattgaagaaaatctgaaacaattgtaagcagcaatccacacctccccagcaatgactcaatttactaaccccattgacagaaaatgtgagcatcttttttagatgtcatgatgataggtggagtattcttaattattgctttcagcaaaccggtgcccataaagtgtttcccattaaatcaatgagaggcattaaggctgagattaaacggttgaacttgaactagataattctagcggaaagaattgctctttttattacgtcgt

SEQ ID NO: 4 - DNA, 1000 bp, Pichia pastoris
aggctctgcgcaaggcaactgagaaattgaatagtggtttcaagcccgctgactttttgtattatctcaatgtcggtgtttcacagtccccagaagggggctttgccttcaagggagacggaagagacatcgtcaaccctggggagaagtatttcaaatggcgcaagttcgctaatttttacgattaagcagtgctgtatggggtagttaataaatcgggaatatccttctgacgtgactgtaacaaatctctttttacgtggtgcgcatactggacagaggcagagtctcaatttcttcttttgagacaggctactacagcctgtgattcctcttggtacttggatttgcttttatctggctccgttgggaactgtgcctgggttttgaagtatcttgtggatgtgtttctaacactttttcaatcttcttggagtgagaatgcaggactttgaacatcgtctagctcgttggtaggtgaaccgttttaccttgcatgtggttaggagttttctggagtaaccaagaccgtcttatcatcgccgtaaaatcgctcttactgtcgctaataatcccgctggaagagaagttcgaacagaagtagcacgcaaagctcttgtcaaatgagaattgttaatcgtttgacaggtcacactcgtgggctatgtacgatcaacttgccggctgttgctggagagatgacaccagttgtggcatggccaattggtattcagccgtaccactgtatggaaaatgagattatcttgttcttgatctagtttcttgccattttagagttgccacattcgtaggtttcagtaccaataatggtaacttccaaacttccaacgcagataccagagatctgccgatccttccccaacaataggagcttactacgccatacatatagcctatctattttcactttcgcgtgggtgcttctatataaacggttccccatcttccgtttcatactacttgaattttaagcactaaa

SEQ ID NO: 5 - DNA, 1000 bp, Pichia pastoris
caaacttaaccgaccgttcttccatccgtttattaatatacacacctatgaactgagccaggttttcaggtctctgtgactctctatacattgacggaacaacatccgttcagtctcatccaattgcagcccaaactctgagtttagcaattgcaaatggttattatctgacgagtaatcgttgatggcacatgccctctgtttgaacatctcttgaacaatagccatcagttctgtgtcattaaacatgcttccccatttcactgacagtttgtagaaatagggcaacaattgatgcaaatcgattttcaacgcattggttttgatagcattgatgatcttggagctgtaaaagtccggctggataagctcaatgaaataggttggttgatctggatcttcttttgggtcattttgttcgctctgtatttcacaaattgccagaatctctgccaaccacagtggtaggtccaacttggtgttctgaatcacaggcttccccgggttgttctctaaataaccgaggcccggcacagaaatcgtaaaccgacacggtatcttttgtccgtccgccagtatctcatcaaggtcgtagtagcccatgatgagtatcaaaggggatttggttatgcgatgcaacgagagattgtttatcccagatgctgatgtaaaaaccttaaccagcgtgacagtagaaataagacacgttaaaattacccgcgcttccctaacaattggctctgcctttcggcaagtttctaactgccctcccctctcacatgcaccacgaacttaccgttcgctcctagcagaaccaccccaaagtttaatcaggaccgcattttagcctattgctgtagaaccccacaacataacctggtccagagccagccctttatatatggtaaatcccgtttgaacttcgaagtggaatcggaatttttacatcaaagaaactgatactgaaacttttggcttcgacttggactttctcttaatc

SEQ ID NO: 6 - DNA, 1000 bp, Pichia pastoris
gtaaataagttaaagtttaaaaaggaaaggatgcaaaaaatatccttgaaggcaacgaatattttgaaatccccgatgccaaataaatgctatcacttaaagagcacaatagaggtggaaaaagaaaaacttggtcaagctaagggttagcaagtttctgtttgtgataatcagggagaaggtgtcagaaaaaacatgattatgtaagtggtgttaggagccgttaaagcattctgtcggccaatagcaagcccgccttttgtcatctttttgcggtttctctgtgtgagacactaatcacctttgtaagacatcgggaaaaccgttgcgcaaaatgagatagagattgttctcgatagaggagcgtagtagcctctccagcctgctttagcaacataatagaaaagaaatatgcgttgcctagggaggctacgtatgcccagcataaacgagtgtttaccttacttcgcacgagcagtagccactaagatcattataaactcacctattgtcttcatgctgtgctccgcgtatttgtctgttcagggtgtcatttctcgtcatgagaatctgattgatgactatgcgagattacccctggattttttttgatcccgtaacgcgaacttgaacattgactttgatatggcaatgggccctaatatgccctaatatgccctaagcttaacaattgacttctgttctctggcagactccacagaaaactggttgacaggtctaatttctttttgaatcatttccggtgattcattttgatgcttagagtgagtcatgggttctttatccgcattcttcttcgcgtctgctgtgcttaataatagcctactaaaaatgtggggagcctcttaccttatgtctataaaaacaagcacatgactatgccatcgccttcatagttgttctgcgggtttttgcttgttttatgaccgtagagaccaaccaatttacatatctacagggtagcacattcgataagaaa

SEQ ID NO: 7 - DNA, 1000 bp, Pichia pastoris
gaagggctacaggttgttcgagtcaaccaagaaaaaaatgtctccattccattaccttcagaagtctgtgatgtgagattcagtagcaacgaaactacacccatagtcagaccaaatgaaaccagtcaagacttttcaatctggctcaaagaccagccaggaatcagagagtttttacaaaattcgaccatcgcacttggatctagactcaatctcttaagcaatgtaaatattgagatacatggggagacagtgaattataccttcacagaaatcgaacagaggagacaattagaactgaattacagacaacaccttcttcaatattcagcagtggaaggaggactactgggtgggaaaagaacagaagtcaatctggtaaatatggctgaagcccctgcaactacagagtcatttgccaagttttccaaggacgttctggatcttgttcgtatactaagttgtacatagagtgaatataagaacaggggcccagttaagactagatctatcaatactgtaatctagactgaataaacctgaatggcaaagaaacaccaaatggagatttccgaggtagtatcgaccgcacttacgagggcggatatgtgtcctcctgatgtatagttacgtcataaagtattgatgcctagaccatttcaatttcgtagtcatctattcgtgaaaagaggcaaggctgattgttcaatttggcaatgatgagccaacagtgcttaaaactggacaaaacttagatcaaatattcaccgttgtaaaacacagttcctctcgtcttcattttagcccatttgcacaaaaccccaacttttacattccggaaaaaaaatgctcctccacctagatgcagagtgtaccgctcaaagaaccctcgatgagtttcgaccatcttcaccaagtgaaataatatttatagtgagggaaagaacatttttttccctgttcgtttctttaccagttaactactacagaatcttctaaa

SEQ ID NO: 8 - DNA, 1000 bp, Pichia pastoris
tggatctggatgtagatgcaactgcccgaaaaaatacaaagaattagaagatagtcccagctgctgtattggcagatggatggtattaactaacgataagtataaaggcgaaaaatacctagataaatactcaatggccgaagaggtcaagcagactctaagcaagggtgaaaaactaaacgttaaagagatattgaagaggcaccacaagtatccaacatgagaagagaacccagaaagagtcaaaatacaaactcgaaaacataccgattggcagaataccagccatacattacatttgatactaatatacataaaatacactaacctccgaaaccatacaaggtacgtccttgtcttttcaaagcgtagacgacatccagagaagtaacagtctttctcttggcatgctcagtgtaagtaacagcatctctaatgacgttctctaagaaagtcttcagcacagctctgacttcttcgtagatcaaagcggaaatacgcttaacaccacctcttctggccaatcttctgatagctggctttgtgataccttgaatgttgtctctaagaatctttctgtgacgcttagcaccggattttcctagaccttttccaccttttcctctaccagacatatttattgattatttgtttatgggtgagtctagaaaaggacgcactcgtcttgtatttatagatgaaaagagttaaggtggacaatgcagtgccaaaccgtaatgttgatacgacacggtacgcgatgaactgagccgtactcctagaggcagagcgtgcgtaaatttgaaactgtaagaacatgtcccatttctatgctaccagaactcataataaacttgcatcccatttcagtcgggagtgtcgcagtgcgaaatactgttggcactgatggcaaaaagtgccaaatcgttatctatgggagactcttataaatatccagatcctccccctcctgcttcttcttgtgtctatcgtagtaaaa

SEQ ID NO: 9 - DNA, 1000 bp, Pichia pastoris
gatcgaggacatggtgttttttttttttatagaagtatcatactaagtgtacttttcacttgcttatcctcttttctacctcaccctcataagcaggaaattcttgacaatcgcaagagtaagcgtgcactacacagccatcggcaacaccgaatttcaccttacagccagtttgtatctcccttaaatatcgtattcgattaatatacactacattacacttaggatctttcacctctcagtcttctagctaacaggatatccttcttttggatagtaactctcttagcgtgaatagcacacaagttagtatcttcgaacaaggaaaccaagtaagcttcgacggattcttgcaaagcaccgatggcagaagattggaatctcaggtcagtcttgaagtcctgagcaatttctctgaccaatctttggaaaggcagctttctgataagcaactcagtagacttttggaatcttctgatttctctcagagcaacggtacctggcttatatctgtggggcttcttgacacctccagcagcagatggagcggattttctggcagccttggaagccaattgctttcttggggctttaccaccagtggattttcttgctgtttgtttagttctagccatttttactacgatagacacaagaagaagcaggagggggaggatctggatatttataagagtctcccatagataacgatttggcactttttgccatcagtgccaacagtatttcgcactgcgacactcccgactgaaatgggatgcaagtttattatgagttctggtagcatagaaatgggacatgttcttacagtttcaaatttacgcacgctctgcctctaggagtacggctcagttcatcgcgtaccgtgtcgtatcaacattacggtttggcactgcattgtccaccttaactcttttcatctataaatacaagacgagtgcgtccttttctagactcacccataaacaaataatcaataaat

SEQ ID NO: 10 - DNA, 1000 bp, Pichia pastoris
ttccatattacttcagcaaatacaagtacaaatcacttgactcgtatcagttcttggataccctttatgagtttttctcagataaacatgaaattttagacaaagttgactgggaaacttggttgtacaagtttggattaccaccaaagccaaagtttgatacctcgctagttgatgaatgctatgatttagctgccaaatgggttgatgtcaccaagaaggatagcaaagatcttttgaagaaaactttcagctcagatgatatttctaatttcacgggtaaccaaactaacgtcttccttgatactttagtatcttatcaaggagtggaaggtttcctgtggaattccaaagaaggggaacaagctttgacgtttatgagagagagctatagcgtttatgacgactccaagaatgcagaagtcattttccgctggtacagactacaattaacagggagaagcaagcagtactaccagcgtctggccgattggctgggaacaatcggacgaatgaaatttgttcgaccatcttatcgaatgctcaacgatgtggaccctcaactggccaaggacacattcttgaagtttgagccaatctaccatccgatctgtcgatcaatgatccgcaaggacttacacttgtagagaaaaaaggtatgtggggtatacgtaagtacgttaagtatgccaaaaacatcacaatagacaatacgccctacaacagaacgtcaagttgtacgcgagcaccgttaaatcacacgtaacatccaacacctttctttggtagggcatagccccaggtggcaccacgtgcataaaccattttacaccccaacacccaccaatcctcgccctctggcatttgctcaaattttttaaccagcttctgattacataggtaaccagttcaattcataggtaagtcaacgccgaacaacaagggaaatcacccatccgctcacatcagtccagttgaagactaacattaaaagacaaaa

SEQ ID NO: 11 - DNA, 1000 bp, Pichia pastoris
tggtaatcaactcactatttcattcatgtcaacagccccgaaaacgataattaatagacaaccccaatcatatttagtgagttttcggattaaagcttgttcgcgttccggttgatgatggtttcaagaaaatgctgagctcgctcttatactgggtcccttgaaatgatatgcatatgttgggaatacgctaatgtactttgacagatattgcttctccttgtagcaaattgacagtttcgtttgcaactgtaacacttggtgatcgatatttggataaacacaattactattttggagttacaaccagaattcgtcttaatgtttcgcatccttgttcaaagactaaaacttcttcgatttcgaatttgtcttaagtattgactagtcgggctcaaagagcaacactagctggaaacggctcaggatcactttcgttttttttctagaaaatgaggcaattgtaggactgggtctctttatctgcaatttgtgtaagctggtttactgttctcaacaaaatagaagtgaaccgtccgtgatgtaaaatgagactactccgttgaatcgcaacaagtattatatcctagcttaaggtgattcttaactttggagcaaaaatatcgtgtaacaacgccggctcagtcaatcttctttgaattaacactgcacctctatcttgaacactatctacatgagtgtgcaaccagaaagaatgcaaagattaattttcttacccacaatgtggtccgatccacaattctagtgaattcctaacatgtttagtaccaacgtttgaacaacagatacatcacattgaaaaaaaggattgagaataataatcaaattttcagcattatatagtaccacgaaactaaatcgctttggaaggagaaacattttcaagctgttaaactggatttatccaaaatagttagtttgcacaagtttaaaaggaggtgtctaacaggtggggaaaaatcagttaattgagttttta

SEQ ID NO: 12 - DNA, 1000 bp, Pichia pastoris
cagggggcagttacttcattatatgtagtaagttgtctaataacactttagaattgagggttgtactaaccaaacagacactgttgcaagttatggtgacaaggttgctttcaagccctgatactaaagtggttcatatttgcatgagtggttcgtatccggaggatcatctacagaacgtgctaaaatcattatcttttggtgacgaaaaaaagaagttaccattggatgacaagacaaagaatactattttagatagtatttggctggcttaccctgacgatctgaatgagtcgtacgaacaattggagaaacttcaagaagagaattcagcgggtctctcaaaactgatgattgttattcaagatttggatgatatggctgagttatacgccttcagagatttcacatcaggtaagtttacactctgaaattttgattacaaaatatatactaacacatttagcctgtgctacattgatgaatttcatgcttaaattaagaaaaatcagtcaactgggagctacggtcatagttactaatatcaatcatgactctggagtgtctatgatattctcctacatagccaagttttacgacaataaactaacgttcagctttcacaaaggctcaatacttttagagatacgtcctctaacgatatcaaccgaacttcagctcagcactactacactctctatcaacccacaaacgatgtaccacatgcttttccccagctctgaaaatgcccttatcagcacgtgattaaagatgagggctcgctgacaagatgtgactagactgccacctttacaccctcagagaagacaaacgtctcatttcgcggttagtaaggttaacccacaaattttcaacgtgtactacccaagagctctctgtctgccatgggcgcgcgcacactccctggtgtgcgaatccaaccaaagtatgaaaaaaaaaaaccattacttcaaagttttctttcaacacacaaaagaag

SEQ ID NO: 13 - DNA, 1000 bp, Pichia pastoris
gtatttgacaggttggggagcaaataagtgatgatgtcccatgaaagtagaaaatggctagtagaaggcaaaaatttgaaattcttagagtcaaatagttagactccaagttctaatccacatttggtcagtttcatagcatccagagcttttgccactggtgaacatatctacccattgcgatgcaacaagtcactgaaagcctaaaacggagattcccctatcttacagcctcgttcaaaaaaactgctaccgtttatctgctatggccgatgtgaggatgcgctcatgcccaagagtccaactttatcaaaaacttgacccgtcatacaggctctagatcaagaagcaaacttaatctcagcatctggttacgtaactctggcaaccagtaacacgcttaaggtttggaacaacactaaactaccttgcggtactaccattgacactacacatccttaattccaatcctgtctggcctccttcaccttttaaccatcttgcccattccaactcgtgtcagattgcgtatcaagtgaaaaaaaaaaaattttaaatctttaacccaatcaggtaataactgtcgcctcttttatctgccgcactgcatgaggtgtccccttagtgggaaagagtactgagccaaccctggaggacagcaagggaaaaatacctacaacttgcttcataatggtcgtaaaaacaatccttgtcggatataagtgttgtagactgtcccttatcctctgcgatgttcttcctctcaaagtttgcgatttctctctatcagaattgccatcaagagactcaggactaatttcgcagtcccacacgcactcgtacatgattggctgaaatttccctaaagaatttctttttcacgaaaattttttttttacacaagattttcagcagatataaaatggagagcaggacctccgctgtgactcttcttttttttcttttattctcactacatacattttagttattcgccaac

SEQ ID NO: 14 - DNA, 1000 bp, Pichia pastoris
attgtttatagcctataatcgcagactttgttaacccgtaggaataatcctaccactagaattagatcttccaaccatacatagcgtgtactacaacttaagctggtcctcttcttttatcattcgcgcggctctatctcatctacacctccattgaactaatggaaagcaaatacgccgaaaaatatcaagatcgattgattcttggagatgatggcgatgaggacgaattgtttgacgagctggaaaaagatattgaggatcaattcttggccaaatacagagcagagagaatccaacagttaaaacaggagattaccaagatcaaggaccatagttcaaacatcaacctcaatgaccacggtaacatgaaaacaatagatactgatgacgaactattgaaagaaactgttgatagcgaacgtgttgtgatccatttctttaacccatcgtttagcacttgccgtatcatggatgagaagctgtctataatcagcaccaaacatattggaacgcgttttttcagaattgaagcacatagagctccatttttagttgcaaagcttggtatcaaagtgcttccatgtgttgtattgtactacaaaggattagaaagggatagaattgtcggatttgacagattaagtaattctcagaccaattttgagctagaagctttagaggagttactcttagatagtggaattgtggaacgaagaactgtcgattttagcaacctgagaaacaaggtccaaaacaaggtggatcagtcaaaatcagactcagaaagtgatctagatatgtgatagatggcggatggcaggttcattctagtgtttcacgtgacacacgtgagcgtttaagggcacacaccctgactgacgcgcgaacatctaatctgttccgcatgaaaaaaaaaaactacctcgacgaaattctcttctagacagtttttacattggtaagaaagaagcattcacgtattgccgacgaagccaaa

SEQ ID NO: 15 - DNA, 939 bp, Pichia pastoris
gatctaacatccaaagacgaaaggttgaatgaaacctttttgccatccgacatccacaggtccattctcacacataagtgccaaacgcaacaggaggggatacactagcagcagaccgttgcaaacgcaggacctccactcctcttctcctcaacacccacttttgccatcgaaaaaccagcccagttattgggcttgattggagctcgctcattccaattccttctattaggctactaacaccatgactttattagcctgtctatcctggcccccctggcgaggttcatgtttgtttatttccgaatgcaacaagctccgcattacacccgaacatcactccagatgagggctttctgagtgtggggtcaaatagtttcatgttccccaaatggcccaaaactgacagtttaaacgctgtcttggaacctaatatgacaaaagcgtgatctcatccaagatgaactaagtttggttcgttgaaatgctaacggccagttggtcaaaaagaaacttccaaaagtcggcataccgtttgtcttgtttggtattgattgacgaatgctcaaaaataatctcattaatgcttagcgcagtctctctatcgcttctgaaccccggtgcacctgtgccgaaacgcaaatggggaaacacccgctttttggatgattatgcattgtctccacattgtatgcttccaagattctggtgggaatactgctgatagcctaacgttcatgatcaaaatttaactgttctaacccctacttgacagcaatatataaacagaaggaagctgccctgtcttaaacctttttttttatcatcattattagcttactttcataattgcgactggttccaattgacaagcttttgattttaacgacttttaacgacaacttgagaagatcaaaaaacaactaattattcgaaacg

SEQ ID NO: 16 - DNA, 1001 bp, Pichia pastoris
catgttggtattgtgaaatagacgcagatcgggaacactgaaaaataacagttattattcgagatctaacatccaaagacgaaaggttgaatgaaacctttttgccatccgacatccacaggtccattctcacacataagtgccaaacgcaacaggaggggatacactagcagcagaccgttgcaaacgcaggacctccactcctcttctcctcaacacccacttttgccatcgaaaaaccagcccagttattgggcttgattggagctcgctcattccaattccttctattaggctactaacaccatgactttattagcctgtctatcctggcccccctggcgaggttcatgtttgtttatttccgaatgcaacaagctccgcattacacccgaacatcactccagatgagggctttctgagtgtggggtcaaatagtttcatgttccccaaatggcccaaaactgacagtttaaacgctgtcttggaacctaatatgacaaaagcgtgatctcatccaagatgaactaagtttggttcgttgaaatgctaacggccagttggtcaaaaagaaacttccaaaagtcggcataccgtttgtcttgtttggtattgattgacgaatgctcaaaaataatctcattaatgcttagcgcagtctctctatcgcttctgaaccccggtgcacctgtgccgaaacgcaaatggggaaacacccgctttttggatgattatgcattgtctccacattgtatgcttccaagattctggtgggaatactgctgatagcctaacgttcatgatcaaaatttaactgttctaacccctacttgacagcaatatataaacagaaggaagctgccctgtcttaaacctttttttttatcatcattattagcttactttcataattgcgactggttccaattgacaagcttttgattttaacgacttttaacgacaacttgagaagatcaaaaaacaactaattattcgaaacg

SEQ ID NO: 17 - DNA, 34 bp, Artificial Sequence
  Description of Artificial Sequence: Synthetic primer
  modified_base (1)..(3): a, c, t, g, unknown or other
  modified_base (10)..(10): a, c, t, g, unknown or other
nnnggtctcnatccacgagtttctggaccgtatc

SEQ ID NO: 18 - DNA, 32 bp, Artificial Sequence
  Description of Artificial Sequence: Synthetic primer
  modified_base (1)..(3): a, c, t, g, unknown or other
nnnggtctctatccggaaaacgttaagagatg

SEQ ID NO: 19 - DNA, 36 bp, Artificial Sequence
  Description of Artificial Sequence: Synthetic primer
  modified_base (1)..(3): a, c, t, g, unknown or other
nnnggtctctatccctctactaaattgccccaagtg

SEQ ID NO: 20 - DNA, 38 bp, Artificial Sequence
  Description of Artificial Sequence: Synthetic primer
  modified_base (1)..(3): a, c, t, g, unknown or other
  modified_base (10)..(10): a, c, t, g, unknown or other
nnnggtctcnatccgatggagactcagtatgatggggc

SEQ ID NO: 21 - DNA, 37 bp, Artificial Sequence
  Description of Artificial Sequence: Synthetic primer
  modified_base (1)..(3): a, c, t, g, unknown or other
  modified_base (10)..(10): a, c, t, g, unknown or other
nnnggtctcnatccagtatgatggggcaaggaaaacg

SEQ ID NO: 22 - DNA, 34 bp, Artificial Sequence
  Description of Artificial Sequence: Synthetic primer
  modified_base (1)..(3): a, c, t, g, unknown or other
  modified_base (10)..(10): a, c, t, g, unknown or other
nnnggtctcnatcctggagacccttaacaggtcg

SEQ ID NO: 23 - DNA, 31 bp, Artificial Sequence
  Description of Artificial Sequence: Synthetic primer
  modified_base (1)..(3): a, c, t, g, unknown or other
  modified_base (10)..(10): a, c, t, g, unknown or other
nnnggtctcnatccgttgggaactgtgcctg

SEQ ID NO: 24 - DNA, 35 bp, Artificial Sequence
  Description of Artificial Sequence: Synthetic primer
  modified_base (1)..(3): a, c, t, g, unknown or other
  modified_base (10)..(10): a, c, t, g, unknown or other
nnnggtctcnatccacagtggtaggtccaacttgg

SEQ ID NO: 25 - DNA, 34 bp, Artificial Sequence
  Description of Artificial Sequence: Synthetic primer
  modified_base (1)..(3): a, c, t, g, unknown or other
  modified_base (10)..(10): a, c, t, g, unknown or other
nnncgtctcnatccgtagtagcctctccagcctg

SEQ ID NO: 26 - DNA, 36 bp, Artificial Sequence
  Description of Artificial Sequence: Synthetic primer
  modified_base (1)..(3): a, c, t, g, unknown or other
  modified_base (10)..(10): a, c, t, g, unknown or other
nnnggtctcnatcctgaagcccctgcaactacagag

SEQ ID NO: 27 - DNA, 40 bp, Artificial Sequence
  Description of Artificial Sequence: Synthetic primer
  modified_base (1)..(3): a, c, t, g, unknown or other
  modified_base (10)..(10): a, c, t, g, unknown or other
nnnggtctcnatccgtagacgacatccagagaagtaacag

SEQ ID NO: 28 - DNA, 38 bp, Artificial Sequence
  Description of Artificial Sequence: Synthetic primer
  modified_base (1)..(3): a, c, t, g, unknown or other
  modified_base (10)..(10): a, c, t, g, unknown or other
nnnggtctcnatcctcaggtcagtcttgaagtcctgag

SEQ ID NO: 29 - DNA, 35 bp, Artificial Sequence
  Description of Artificial Sequence: Synthetic primer
  modified_base (1)..(3): a, c, t, g, unknown or other
  modified_base (10)..(10): a, c, t, g, unknown or other
nnnggtctcnatcctgtggaattccaaagaagggg

SEQ ID NO: 30 - DNA, 38 bp, Artificial Sequence
  Description of Artificial Sequence: Synthetic primer
  modified_base (1)..(3): a, c, t, g, unknown or other
  modified_base (10)..(10): a, c, t, g, unknown or other
nnnggtctcnatccgtccgtgatgtaaaatgagactac

SEQ ID NO: 31 - DNA, 34 bp, Artificial Sequence
  Description of Artificial Sequence: Synthetic primer
  modified_base (1)..(3): a, c, t, g, unknown or other
  modified_base (10)..(10): a, c, t, g, unknown or other
nnnggtctcnatccagtcaactgggagctacggt

SEQ ID NO: 32 - DNA, 31 bp, Artificial Sequence
  Description of Artificial Sequence: Synthetic primer
  modified_base (1)..(3): a, c, t, g, unknown or other
  modified_base (10)..(10): a, c, t, g, unknown or other
nnnggtctcnatccgatgtgaggatgcgctc

SEQ ID NO: 33 - DNA, 39 bp, Artificial Sequence
  Description of Artificial Sequence: Synthetic primer
  modified_base (1)..(3): a, c, t, g, unknown or other
  modified_base (10)..(10): a, c, t, g, unknown or other
nnnggtctcnatcctcaatgaccacggtaacatgaaaac

SEQ ID NO: 34 - DNA, 37 bp, Artificial Sequence
  Description of Artificial Sequence: Synthetic primer
  modified_base (1)..(3): a, c, t, g, unknown or other
  modified_base (10)..(10): a, c, t, g, unknown or other
nnnggtctcnatccaatggaccaaattgttgcaaggt

SEQ ID NO: 35 - DNA, 29 bp, Artificial Sequence
  Description of Artificial Sequence: Synthetic primer
  modified_base (1)..(3): a, c, t, g, unknown or other
nnnggtctccatccctttgttgagcaaca

SEQ ID NO: 36 - DNA, 28 bp, Artificial Sequence
  Description of Artificial Sequence: Synthetic primer
  modified_base (1)..(3): a, c, t, g, unknown or other
nnnggtctcgatccgcccaaacgaacag

SEQ ID NO: 37 - DNA, 34 bp, Artificial Sequence
  Description of Artificial Sequence: Synthetic primer
  modified_base (1)..(3): a, c, t, g, unknown or other
nnnggtctccatccaaagacgaaaggttgaatga